European Patent Application EP 4 361 262 A2, published May 1, 2024. Title: Polypeptide epitopes of S. aureus and respective monoclonal antibodies for the treatment of infections and immune-diagnosis. Applicant: Alexander Klimka, Oleg Krut, Martin Kroenke. The sequence listing filed with the application follows.

SEQUENCE LISTING (32 sequences)

SEQ ID NO: 1 - protein, 466 aa, Staphylococcus aureus
MTKSVAIIGAGITGLSSAYFLKQQDPNIDVTIFEASNRPGGKIQSYRKDGYMIELGPESYLGRKTIMTELAKDIGLEQDIVTNTTGQSYIFAKNKLYPIPGGSIMGIPTDIKPFVTTKLISPLGKLRAGLDLIKKPIQMQDGDISVGAFFRARLGNEVLENLIEPLMGGIYGTDIDKLSLMSTFPNFKEKEEAFGSLIKGMKDEKNKRLKQRQLYPGAPKGQFKQFKHGLSSFIEALEQDVKNKGVTIRYNTSVDDIITSQKQYKIVYSNQQEDVFDGVLVTTPHQVFLNWFGQDPAFDYFKTMDSTTVATVVLAFDEKDIENTYDGTGFVIARTSDTDITACTWTSKKWPFTTPEGKVLIRAYVGKPGDTVVDDHTDNELVSIVRRDLSQMMTFKGDPEFTIVNRLPKSMPQYHVGHIQQIRQIQAHIKQTYPRLRVTGASFEAVGLPDCITQGKVAAEEVIAEL

SEQ ID NO: 2 - protein, 253 aa, Staphylococcus aureus
MRTPIIAGNWKMNKTVQEAKDFVNALPTLPDSKEVESVICAPAIQLDALTTAVKEGKAQGLEIGAQNTYFEDNGAFTGETSPVALADLGVKYVVIGHSERRELFHETDEEINKKAHAIFKHGMTPIICVGETDEERESGKANDVVGEQVKKAVAGLSEDQLKSVVIAYEPIWAIGTGKSSTSEDANEMCAFVRQTIADLSSKEVSEATRIQYGGSVKPNNIKEYMAQTDIDGALVGGASLKVEDFVQLLEGAK

SEQ ID NO: 3 - protein, 306 aa, Staphylococcus aureus
MIRNRVMNSVVNKYLLHNRSIMFKNDQDVERFFYKREIENRKKHKQPSTLNVKANLEKLSLDDMQVFRFNFRHQIDKKILYIHGGFNALQPSPFHWRLLDKITLSTLYEVVLPIYPKTPEFHIDDTFQAIQRVYDQLVSEVGHQNVVVMGDGSGGALALSFVQSLLDNQQPLPNKLYLISPILDATLSNKDISDALIEQDAVLSQFGVNEIMKKWANGLPLTDKRISPINGTIEGLPPVYMFGGGREMTHPDMKLFEQMMLQHHQYIEFYDYPKMVHDFPIYPIRQSHKAIKQIAKSIDEDVTQNN

SEQ ID NO: 4 - protein, 12 aa, Staphylococcus aureus
KNDQDVERFFYK

SEQ ID NO: 5 - protein, 16 aa, Staphylococcus aureus
HTDNELVSIVRRDLSQ

SEQ ID NO: 6 - protein, 108 aa, Staphylococcus aureus
NKKAHAIFKHGMTPIICVGETDEERESGKANDVVGEQVKKAVAGLSEDQLKSVVIAYEPIWAIGTGKSSTSEDANEMCAFVRQTIADLSSKEVSEATRIQYGGSVKPN

SEQ ID NO: 7 - protein, 15 aa, Staphylococcus aureus
NKKAHAIFKHGMTPI

SEQ ID NO: 8 - protein, 11 aa, Staphylococcus aureus
QLKSVVIAYEP

SEQ ID NO: 9 - protein, 15 aa, Staphylococcus aureus
ANEMCAFVRQTIADL

SEQ ID NO: 10 - protein, 20 aa, Staphylococcus aureus
SSKEVSEATRIQYGGSVKPN

SEQ ID NO: 11 - protein, 130 aa, synthetic construct
  REGION 1..130: note = triepitope peptide sequence
TDNELVSIVRRDKAHAIFKHGMTPIICVGETDEERESGKANDVVGEQVKKAVAGLSEDQLKSVVIAYEPIWAIGTGKSSTSEDANEMCAFVRQTIADLSSKEVSEATRIQYGGSVKPNKNDQDVERFFYK

SEQ ID NO: 12 - protein, 118 aa, synthetic construct
  REGION 1..118: note = diepitope peptide sequence
TDNELVSIVRRDKAHAIFKHGMTPIICVGETDEERESGKANDVVGEQVKKAVAGLSEDQLKSVVIAYEPIWAIGTGKSSTSEDANEMCAFVRQTIADLSSKEVSEATRIQYGGSVKPN

SEQ ID NO: 13 - protein, 130 aa, synthetic construct
  REGION 1..130: note = diepitope peptide sequence
TDNELVSIVRRDKAHAIFKHGMTPIICVGETDEERESGKANDVVGEQVKKAVAGLSEDQLKSVVIAYEPIWAIGTGKSSTSEDANEMCAFVRQTIADLSSKEVSEATRIQYGGSVKPNTDNELVSIVRRD

SEQ ID NO: 14 - protein, 118 aa, synthetic construct
  REGION 1..118: note = diepitope peptide sequence
KAHAIFKHGMTPIICVGETDEERESGKANDVVGEQVKKAVAGLSEDQLKSVVIAYEPIWAIGTGKSSTSEDANEMCAFVRQTIADLSSKEVSEATRIQYGGSVKPNTDNELVSIVRRD

SEQ ID NO: 15 - protein, 10 aa, Mus musculus
GYTFTDYSMH

SEQ ID NO: 16 - protein, 17 aa, Mus musculus
WIDTETGEPTFADDFKG

SEQ ID NO: 17 - protein, 11 aa, Mus musculus
PLLRLSFAMDS

SEQ ID NO: 18 - protein, 15 aa, Mus musculus
SASENLDIYGNSFMH

SEQ ID NO: 19 - protein, 7 aa, Mus musculus
RASKLES

SEQ ID NO: 20 - protein, 9 aa, Mus musculus
QQTSEDPRT

SEQ ID NO: 21 - protein, 6 aa, Mus musculus
SRYWIE

SEQ ID NO: 22 - protein, 17 aa, Mus musculus
EILPGSGSTNYNEKFKG

SEQ ID NO: 23 - protein, 12 aa, Mus musculus
FYSGNFVGPVDY

SEQ ID NO: 24 - protein, 16 aa, Mus musculus
KSSQSLSDSDGKTYLN

SEQ ID NO: 25 - protein, 7 aa, Mus musculus
LVSKVDS

SEQ ID NO: 26 - protein, 9 aa, Mus musculus
WQGTHFPFT

SEQ ID NO: 27 - protein, 10 aa, Mus musculus
GFTFSAYWMN

SEQ ID NO: 28 - protein, 19 aa, Mus musculus
EIRMKSNNYATHYAESVKG

SEQ ID NO: 29 - protein, 7 aa, Mus musculus
YKYDGAY

SEQ ID NO: 30 - protein, 10 aa, Mus musculus
SASSTVNYMH

SEQ ID NO: 31 - protein, 7 aa, Mus musculus
DTSKLAS

SEQ ID NO: 32 - protein, 8 aa, Mus musculus
HQRSSYPT